European Patent Specification EP 3 501 272 B1, published March 1, 2023. Title: Mice Expressing A Limited Immunoglobulin Light Chain Repertoire. Applicant: BABB, Robert MCWHIRTER, John MACDONALD, Lynn STEVENS, Sean DAVIS, Samuel BUCKLER, David R. HOSIAWA, Karolina A. MURPHY, Andrew J. The sequence listing filed with the application follows.

SEQUENCE LISTING (49 sequences)

SEQ ID NO: 1 - DNA, 3155 bp, Artificial Sequence
  Synthetic
ggcgcgccgtagctttgaattttaaacatctatttgacaagaaatgcatagttccttctctttaaaataatgtaatgtttctttcaagaataagcttggtttgatgcctctctccccaacatgatagaagtgtagcataaatctatgaaaaattccatttccctgtgcctacaacaactacctgggattgaaaacttcttcccttgctctagtcctttcttctacacctacttccacatcatctgtgactcaaaacaatacttgtcaggaaagatcccggaaagagcaaaaaagacttccttagaggtgtcagagattcctatgccactatctgtcatctctagaaggggttgtgagtatgaggaagagcagagcttgtaaattttctacttgctttgacttccactgtatttcctaacaacaacaaccacagcaacacccataacatcacaggacaaacttctagtacttccaaggctttagtctcagtaaatcttctctacctccatcacagcagctagaaggtttgatactcatacaaatagtactgtagctttctgttcataattggaaaaatagacaagacccaatgtaatacaggctttccttcagccagttagcgttcagtttttggatcaccattgcacacatatacccagcatatgtctaatatatatgtagaaatccgtgaagcaagagttataatagcttgtgttttctattgtattgtattttcctcttatatcatcttcttcttcgttcattaaaaaaaaaccgttcaagtaggtctaaattaattattggatcataagtagataaaatattttatttcataacacattgacccgatgaatatgtttctttgccagacatagtcctcatttccaaggtaacaagcctgaaaaaattatactggagcaagtcaacaggtaatgatggtagcttttccttattgtcctggggcaagaataagacaaaagataacagggtagaataaagattgtgtaagaaagaaggacagcaacaggacatgggaaccttttatagagtaacattttgataatggatgatgagaattaatgagttagacagggatgggtgggaatgattgaaggtgtgagtactttagcacagattaagaccaaatcattaggatttaaagagttgtgtagagttagtgaaggaaaagccttagaattaaatttggctgcggataaaacattcttggattagactgaagactcttttctgtgctaagtaagtatatttatgataatgatgatgactgtagtgctgaatatttaataaataaaaacaaaattaattgccgcatacataatgtcctgaatactattgtaaatgttttatcttatttcctttaaactgtctacagcactataaggtaggtaccagtattgtcacagttacacagatatggaaaccgagacacagggaagttaagttacttgatcaatttcaagcaatcggcaagccatggagcatctatgtcagggctgccaggacatgtgactgtaaacagaagtttttcactttttaactcaaagagggtatgtggctgggttaatggaaagcttcaggaccctcagaaaacattactaacaagcaaatgaaaggtgtatctggaagattaagttttaacagactcttcatttccatcgatccaataatgcacttagggagatgactgggcatattgaggataggaagagagaagtgaaaacacagctttttatattgttcttaacaggcttgtgccaaacatcttctgggtggatttaggtgattgaggagaagaaagacacaggagcgaaattctctgagcacaagggaggagttctacactcagactgagccaacagacttttctggcctgacaaccagggcggcgcaggatgctcagtgcagagaggaagaagcaggtggtctttgcagctgaaagctcagctgatttgcatatggagtcattatacaacatcccagaattctttaagggcagctgccaggaagctaagaagcatcctctcttctagctctcagagatggagacagacacactcctgctatgggtgctgctgctctgggttccaggtgagggtacagataagtgttatgagcaacctctgtggccattatgatgctccatgcctctctgttcttgatcactataattagggcatttgtcactggttttaagtttccccagtcccctgaattttccattttctcagagtgatgtccaaaattattcttaaaaatttaaatgaaaaggtcctctgctgtgaaggcttttaaagatatataaaaataatctttgtgtttatcattccaggtgccagatgtgacatccagatgacccagtctccatcctccctgtctgcatctgtaggagacagagtcaccatcacttgccgggcaagtcagagcattagcagctatttaaattggtatcagcagaaaccagggaaagcccctaagctcctgatctatgctgcatccagtttgcaaagtggggtcccatcaaggttcagtggcagtggatctgggacagatttcactctcaccatcagcagtctgcaacctgaagattttgcaacttactactgtcaacagagttacagtacccctccgatcaccttcggccaagggacacgactggagattaaacgtaagtaatttttcactattgtcttctgaaatttgggtctgatggccagtattgacttttagaggcttaaataggagtttggtaaagattggtaaatgagggcatttaagatttgccatgggttgcaaaagttaaactcagcttcaaaaatggatttggagaaaaaaagattaaattgctctaaactgaatgacacaaagtaaaaaaaaaaagtgtaactaaaaaggaacccttgtatttctaaggagcaaaagtaaatttatttttgttcactcttgccaaatattgtattggttgttgctgattatgcatgatacagaaaagtggaaaaatacattttttagtctttctcccttttgtttgataaattattttgtcagacaacaataaaaatcaatagcacgccctaagatctagatgcatgctcgagtgccatttcattacctctttctccgcacccgacatagat

SEQ ID NO: 2 - DNA, 28 bp, Artificial Sequence
  Synthetic
aggtgagggtacagataagtgttatgag

SEQ ID NO: 3 - DNA, 27 bp, Artificial Sequence
  Synthetic
tgacaaatgccctaattatagtgatca

SEQ ID NO: 4 - DNA, 21 bp, Artificial Sequence
  Synthetic
gggcaagtcagagcattagca

SEQ ID NO: 5 - DNA, 21 bp, Artificial Sequence
  Synthetic
tgcaaactggatgcagcatag

SEQ ID NO: 6 - DNA, 19 bp, Artificial Sequence
  Synthetic
ggtggagaggctattcggc

SEQ ID NO: 7 - DNA, 17 bp, Artificial Sequence
  Synthetic
gaacacggcggcatcag

SEQ ID NO: 8 - DNA, 23 bp, Artificial Sequence
  Synthetic
tgggcacaacagacaatcggctg

SEQ ID NO: 9 - DNA, 29 bp, Artificial Sequence
  Synthetic
ccattatgatgctccatgcctctctgttc

SEQ ID NO: 10 - DNA, 26 bp, Artificial Sequence
  Synthetic
atcagcagaaaccagggaaagcccct

SEQ ID NO: 11 - DNA, 3166 bp, Artificial Sequence
  Synthetic
ggcgcgccgtagctttgaattttaaacatctatttgacaagaaatgcatagttccttctctttaaaataatgtaatgtttctttcaagaataagcttggtttgatgcctctctccccaacatgatagaagtgtagcataaatctatgaaaaattccatttccctgtgcctacaacaactacctgggattgaaaacttcttcccttgctctagtcctttcttctacacctacttccacatcatctgtgactcaaaacaatacttgtcaggaaagatcccggaaagagcaaaaaagacttccttagaggtgtcagagattcctatgccactatctgtcatctctagaaggggttgtgagtatgaggaagagcagagcttgtaaattttctacttgctttgacttccactgtatttcctaacaacaacaaccacagcaacacccataacatcacaggacaaacttctagtacttccaaggctttagtctcagtaaatcttctctacctccatcacagcagctagaaggtttgatactcatacaaatagtactgtagctttctgttcataattggaaaaatagacaagacccaatgtaatacaggctttccttcagccagttagcgttcagtttttggatcaccattgcacacatatacccagcatatgtctaatatatatgtagaaatccgtgaagcaagagttataatagcttgtgttttctattgtattgtattttcctcttatatcatcttcttcttcgttcattaaaaaaaaaccgttcaagtaggtctaaattaattattggatcataagtagataaaatattttatttcataacacattgacccgatgaatatgtttctttgccagacatagtcctcatttccaaggtaacaagcctgaaaaaattatactggagcaagtcaacaggtaatgatggtagcttttccttattgtcctggggcaagaataagacaaaagataacagggtagaataaagattgtgtaagaaagaaggacagcaacaggacatgggaaccttttatagagtaacattttgataatggatgatgagaattaatgagttagacagggatgggtgggaatgattgaaggtgtgagtactttagcacagattaagaccaaatcattaggatttaaagagttgtgtagagttagtgaaggaaaagccttagaattaaatttggctgcggataaaacattcttggattagactgaagactcttttctgtgctaagtaagtatatttatgataatgatgatgactgtagtgctgaatatttaataaataaaaacaaaattaattgccgcatacataatgtcctgaatactattgtaaatgttttatcttatttcctttaaactgtctacagcactataaggtaggtaccagtattgtcacagttacacagatatggaaaccgagacacagggaagttaagttacttgatcaatttcaagcaatcggcaagccatggagcatctatgtcagggctgccaggacatgtgactgtaaacagaagtttttcactttttaactcaaagagggtatgtggctgggttaatggaaagcttcaggaccctcagaaaacattactaacaagcaaatgaaaggtgtatctggaagattaagttttaacagactcttcatttccatcgatccaataatgcacttagggagatgactgggcatattgaggataggaagagagaagtgaaaacacagctttttatattgttcttaacaggcttgtgccaaacatcttctgggtggatttaggtgattgaggagaagaaagacacaggagcgaaattctctgagcacaagggaggagttctacactcagactgagccaacagacttttctggcctgacaaccagggcggcgcaggatgctcagtgcagagaggaagaagcaggtggtctttgcagctgaaagctcagctgatttgcatatggagtcattatacaacatcccagaattctttaagggcagctgccaggaagctaagaagcatcctctcttctagctctcagagatggagacagacacactcctgctatgggtgctgctgctctgggttccaggtgagggtacagataagtgttatgagcaacctctgtggccattatgatgctccatgcctctctgttcttgatcactataattagggcatttgtcactggttttaagtttccccagtcccctgaattttccattttctcagagtgatgtccaaaattattcttaaaaatttaaatgaaaaggtcctctgctgtgaaggcttttaaagatatataaaaataatctttgtgtttatcattccaggtgccagatgtataccaccggagaaattgtgttgacgcagtctccaggcaccctgtctttgtctccaggggaaagagccaccctctcctgcagggccagtcagagtgttagcagcagctacttagcctggtaccagcagaaacctggccaggctcccaggctcctcatctatggtgcatccagcagggccactggcatcccagacaggttcagtggcagtgggtctgggacagacttcactctcaccatcagcagactggagcctgaagattttgcagtgtattactgtcagcagtatggtagctcaccttggacgttcggccaagggaccaaggtggaaatcaaacgtaagtaatttttcactattgtcttctgaaatttgggtctgatggccagtattgacttttagaggcttaaataggagtttggtaaagattggtaaatgagggcatttaagatttgccatgggttgcaaaagttaaactcagcttcaaaaatggatttggagaaaaaaagattaaattgctctaaactgaatgacacaaagtaaaaaaaaaaagtgtaactaaaaaggaacccttgtatttctaaggagcaaaagtaaatttatttttgttcactcttgccaaatattgtattggttgttgctgattatgcatgatacagaaaagtggaaaaatacattttttagtctttctcccttttgtttgataaattattttgtcagacaacaataaaaatcaatagcacgccctaagatctagatgcatgctcgagtgccatttcattacctctttctccgcacccgacatagat

SEQ ID NO: 12 - DNA, 19 bp, Artificial Sequence
  Synthetic
tccaggcaccctgtctttg

SEQ ID NO: 13 - DNA, 26 bp, Artificial Sequence
  Synthetic
aagtagctgctgctaacactctgact

SEQ ID NO: 14 - DNA, 24 bp, Artificial Sequence
  Synthetic
aaagagccaccctctcctgcaggg

SEQ ID NO: 15 - DNA, 3187 bp, Artificial Sequence
  Synthetic
ggcgcgccgtagctttgaattttaaacatctatttgacaagaaatgcatagttccttctctttaaaataatgtaatgtttctttcaagaataagcttggtttgatgcctctctccccaacatgatagaagtgtagcataaatctatgaaaaattccatttccctgtgcctacaacaactacctgggattgaaaacttcttcccttgctctagtcctttcttctacacctacttccacatcatctgtgactcaaaacaatacttgtcaggaaagatcccggaaagagcaaaaaagacttccttagaggtgtcagagattcctatgccactatctgtcatctctagaaggggttgtgagtatgaggaagagcagagcttgtaaattttctacttgctttgacttccactgtatttcctaacaacaacaaccacagcaacacccataacatcacaggacaaacttctagtacttccaaggctttagtctcagtaaatcttctctacctccatcacagcagctagaaggtttgatactcatacaaatagtactgtagctttctgttcataattggaaaaatagacaagacccaatgtaatacaggctttccttcagccagttagcgttcagtttttggatcaccattgcacacatatacccagcatatgtctaatatatatgtagaaatccgtgaagcaagagttataatagcttgtgttttctattgtattgtattttcctcttatatcatcttcttcttcgttcattaaaaaaaaaccgttcaagtaggtctaaattaattattggatcataagtagataaaatattttatttcataacacattgacccgatgaatatgtttctttgccagacatagtcctcatttccaaggtaacaagcctgaaaaaattatactggagcaagtcaacaggtaatgatggtagcttttccttattgtcctggggcaagaataagacaaaagataacagggtagaataaagattgtgtaagaaagaaggacagcaacaggacatgggaaccttttatagagtaacattttgataatggatgatgagaattaatgagttagacagggatgggtgggaatgattgaaggtgtgagtactttagcacagattaagaccaaatcattaggatttaaagagttgtgtagagttagtgaaggaaaagccttagaattaaatttggctgcggataaaacattcttggattagactgaagactcttttctgtgctaagtaagtatatttatgataatgatgatgactgtagtgctgaatatttaataaataaaaacaaaattaattgccgcatacataatgtcctgaatactattgtaaatgttttatcttatttcctttaaactgtctacagcactataaggtaggtaccagtattgtcacagttacacagatatggaaaccgagacacagggaagttaagttacttgatcaatttcaagcaatcggcaagccatggagcatctatgtcagggctgccaggacatgtgactgtaaacagaagtttttcactttttaactcaaagagggtatgtggctgggttaatggaaagcttcaggaccctcagaaaacattactaacaagcaaatgaaaggtgtatctggaagattaagttttaacagactcttcatttccatcgatccaataatgcacttagggagatgactgggcatattgaggataggaagagagaagtgaaaacacagctttttatattgttcttaacaggcttgtgccaaacatcttctgggtggatttaggtgattgaggagaagaaagacacaggagcgaaattctctgagcacaagggaggagttctacactcagactgagccaacagacttttctggcctgacaaccagggcggcgcaggatgctcagtgcagagaggaagaagcaggtggtctttgcagctgaaagctcagctgatttgcatatggagtcattatacaacatcccagaattctttaagggcagctgccaggaagctaagaagcatcctctcttctagctctcagagatggagacagacacactcctgctatgggtgctgctgctctgggttccaggtgagggtacagataagtgttatgagcaacctctgtggccattatgatgctccatgcctctctgttcttgatcactataattagggcatttgtcactggttttaagtttccccagtcccctgaattttccattttctcagagtgatgtccaaaattattcttaaaaatttaaatgaaaaggtcctctgctgtgaaggcttttaaagatatataaaaataatctttgtgtttatcattccaggtgccagatgtgttgtggtcctcagccggtgctgcatcagccgccggccatgtcctcggcccttggaaccacaatccgcctcacctgcaccctgaggaacgaccatgacatcggtgtgtacagcgtctactggtaccagcagaggccgggccaccctcccaggttcctgctgagatatttctcacaatcagacaagagccagggcccccaggtcccccctcgcttctctggatccaaagatgtggccaggaacagggggtatttgagcatctctgagctgcagcctgaggacgaggctatgtattactgtgctatgcataactcagtgacgcatgtgtttggcagcgggacccagctcaccgttttaagtaagtaatttttcactattgtcttctgaaatttgggtctgatggccagtattgacttttagaggcttaaataggagtttggtaaagattggtaaatgagggcatttaagatttgccatgggttgcaaaagttaaactcagcttcaaaaatggatttggagaaaaaaagattaaattgctctaaactgaatgacacaaagtaaaaaaaaaaagtgtaactaaaaaggaacccttgtatttctaaggagcaaaagtaaatttatttttgttcactcttgccaaatattgtattggttgttgctgattatgcatgatacagaaaagtggaaaaatacattttttagtctttctcccttttgtttgataaattattttgtcagacaacaataaaaatcaatagcacgccctaagatctagatgcatgctcgagtgccatttcattacctctttctccgcacccgacatagat

SEQ ID NO: 16 - DNA, 17 bp, Artificial Sequence
  Synthetic
tgtcctcggcccttgga

SEQ ID NO: 17 - DNA, 20 bp, Artificial Sequence
  Synthetic
ccgatgtcatggtcgttcct

SEQ ID NO: 18 - DNA, 23 bp, Artificial Sequence
  Synthetic
acaatccgcctcacctgcaccct

SEQ ID NO: 19 - DNA, 23 bp, Artificial Sequence
  synthetic
agcagtctgcaacctgaagattt

SEQ ID NO: 20 - DNA, 24 bp, Artificial Sequence
  synthetic
gtttaatctccagtcgtgtccctt

SEQ ID NO: 21 - DNA, 15 bp, Artificial Sequence
  synthetic
cctccgatcaccttc

SEQ ID NO: 22 - DNA, 20 bp, Artificial Sequence
  synthetic
aaaccagggaaagcccctaa

SEQ ID NO: 23 - DNA, 18 bp, Artificial Sequence
  synthetic
atgggaccccactttgca

SEQ ID NO: 24 - DNA, 19 bp, Artificial Sequence
  synthetic
ctcctgatctatgctgcat

SEQ ID NO: 25 - DNA, 21 bp, Artificial Sequence
  synthetic
cagcagactggagcctgaaga

SEQ ID NO: 26 - DNA, 21 bp, Artificial Sequence
  synthetic
tgatttccaccttggtccctt

SEQ ID NO: 27 - DNA, 18 bp, Artificial Sequence
  synthetic
tagctcaccttggacgtt

SEQ ID NO: 28 - DNA, 22 bp, Artificial Sequence
  synthetic
ctcctcatctatggtgcatcca

SEQ ID NO: 29 - DNA, 20 bp, Artificial Sequence
  synthetic
gacccactgccactgaacct

SEQ ID NO: 30 - DNA, 13 bp, Artificial Sequence
  synthetic
ccactggcatccc

SEQ ID NO: 31 - DNA, 19 bp, Artificial Sequence
  synthetic
tgagcagcaccctcacgtt

SEQ ID NO: 32 - DNA, 23 bp, Artificial Sequence
  synthetic
gtggcctcacaggtatagctgtt

SEQ ID NO: 33 - DNA, 18 bp, Artificial Sequence
  synthetic
accaaggacgagtatgaa

SEQ ID NO: 34 - DNA, 22 bp, Artificial Sequence
  synthetic
aagaagcacacgactgaggcac

SEQ ID NO: 35 - DNA, 24 bp, Artificial Sequence
  synthetic
ctcactggatggtgggaagatgga

SEQ ID NO: 36 - DNA, 16 bp, Artificial Sequence
  synthetic
gtaaaacgacggccag

SEQ ID NO: 37 - DNA, 17 bp, Artificial Sequence
  synthetic
caggaaacagctatgac

SEQ ID NO: 38 - protein, 123 aa, Artificial Sequence
  synthetic
DIQMTQSPSSLSASVGDRVTITCRASQSISSYLNWYQQKPGKAPKLLIYAASSLQSGVPSRFSGSGSGTDFTLTISSLQPEDFATYYCQQSYSTPYTFGQGTKLEIKRADAAPTVSIFPPSSE

SEQ ID NO: 39 - protein, 123 aa, Artificial Sequence
  synthetic
DIQMTQSPSSLSASVGDRVTITCRASQSISSYLNWYQQKPGKAPKLLIYAASSLQSGVPSRFSGSGSGTDFTLTISSLQPEDFATYYCQQSYSTPFTFGPGTKVDIKRADAAPTVSIFPPSSE

SEQ ID NO: 40 - protein, 124 aa, Artificial Sequence
  synthetic
EIVLTQSPGTLSLSPGERATLSCRASQSVSSSYLAWYQQKPGQAPRLLIYGASSRATGIPDRFSGSGSGTDFTLTISRLEPEDFAVYYCQQYGSSPRTFGQGTKVEIKRADAAPTVSIFPPSSE

SEQ ID NO: 41 - protein, 123 aa, Artificial Sequence
  synthetic
EIVLTQSPGTLSLSPGERATLSCRASQSVSSSYLAWYQQKPGQAPRLLIYGASSRATGIPDRFSGSGSGTDFTLTISRLEPEDFAVYYCQQYGSSRTFGQGTKVEIKRADAAPTVSIFPPSSE

SEQ ID NO: 42 - protein, 124 aa, Artificial Sequence
  synthetic
EIVLTQSPGTLSLSPGERATLSCRASQSVSSSYLAWYQQKPGQAPRLLIYGASSRATGIPDRFSGSGSGTDFTLTISRLEPEDFAVYYCQQYGSSPWTFGQGTKVEIKRADAAPTVSIFPPSSE

SEQ ID NO: 43 - protein, 124 aa, Artificial Sequence
  synthetic
EIVLTQSPGTLFLSPGERATLSCRASQSVSSSYLAWYQQKPGQAPRLLIYGASSRATGIPDRFSGSGSGTDFTLTISRLEPEDFAVYYCQQYGSSPWTFGQGTKVEIKRADAAPTVSIFPPSSE

SEQ ID NO: 44 - protein, 124 aa, Artificial Sequence
  synthetic
EIVLTQSPGTLSLSPGERATLSCRASQSVSSSYLAWYQQKPGQAPRHLIYGASSRATGIPDRFSGSGSGTDFTLTISRLDPEDFAVYYCQQYGSSPRTFGQGTKVEIKRADAAPTVSIFPPSSE

SEQ ID NO: 45 - protein, 118 aa, Artificial Sequence
  synthetic
EIVLTQSPGTLSLSPGERATLSCRASQSVSSSYLAWYQQKPGQAPRLLIYGASSRATGIPDRFSGSGSGTDFTLTISRLEPEDFAVYYCQQYGSSPRTFGQGTKVEIKRADAAPTVSI

SEQ ID NO: 46 - protein, 124 aa, Artificial Sequence; identical to SEQ ID NO: 42
  synthetic

SEQ ID NO: 47 - protein, 124 aa, Artificial Sequence
  synthetic
EIVLTQSPGTLSLSPGERATLSCRASQSVSSSHLAWYQQKPGQAPRLLIYGASSRATGIPDRFSGSGSGTDFTLTISRLEPEDFAVYYCQQYGSSPPTFGQGTKVEIKRADAAPTVSIFPPSSE

SEQ ID NO: 48 - protein, 124 aa, Artificial Sequence
  synthetic
EIVLTQSPGTLSLSPGERATLSCRASQSVSSSYLAWYQQKPGQAPRLLIYGASSRATGIPDRFSGSGSGTDFTLTISRLEPEDFAVYYCQQYGSSPYTFGQGTKLEIKRADAAPTVSIFPPSSE

SEQ ID NO: 49 - protein, 124 aa, Artificial Sequence
  synthetic
EIVLTQSPGTLSLSPGERATLSCRASQSVSSSYLAWYQQKPGQAPRLLIYGASSRATGIPDRFSGSGSGTDFTLTISRLEPEDFAVYYCQQYGSSIFTFGPGTKVDIKRADAAPTVSIFPPSSE